European Patent Specification EP 3 585 374 B1, published July 19, 2023. Title: COMBINATION THERAPY. Applicant: GENFIT. The sequence listing filed with the application follows.

SEQUENCE LISTING (10 sequences)

SEQ ID NO: 1 - DNA, 25 bp, artificial
  primer
catgctcaacatctcccccttctcc

SEQ ID NO: 2 - DNA, 25 bp, artificial
  primer
gggaaggtgtaatccgtctccacag

SEQ ID NO: 3 - DNA, 20 bp, artificial
  primer
actgggacgacatggaaaag

SEQ ID NO: 4 - DNA, 20 bp, artificial
  primer
catctccagagtccagcaca

SEQ ID NO: 5 - DNA, 20 bp, artificial
  primer
tccccagaaatcatcgagac

SEQ ID NO: 6 - DNA, 20 bp, artificial
  primer
tcagattatgccagggaacc

SEQ ID NO: 7 - DNA, 20 bp, artificial
  primer
tgagtggctgtcttttgacg

SEQ ID NO: 8 - DNA, 20 bp, artificial
  primer
tgggactgatcccattgatt

SEQ ID NO: 9 - DNA, 20 bp, artificial
  primer
cagaacagtcaactttgggg

SEQ ID NO: 10 - DNA, 20 bp, artificial
  primer
acgtggaaaatgaggactgc